European Patent Specification EP 3 623 010 B1, published September 25, 2024. Title: CHIMERIC ANTIGEN RECEPTOR, NUCLEIC ACID, CHIMERIC ANTIGEN RECEPTOR EXPRESSION PLASMID, CHIMERIC ANTIGEN RECEPTOR EXPRESSING CELL, USE THEREOF, AND PHARMACEUTICAL COMPOSITION FOR TREATING CANCER. Applicant: China Medical University Hospital. The sequence listing filed with the application follows.

SEQUENCE LISTING (17 sequences)

SEQ ID NO: 1 - protein, 246 aa, Artificial Sequence
  anti-HLA-G antibody
EVQLQESGGGLVQPKGSLKLSCAAFGFTFNTYAMHWVRQAPGKGLEWVARIRSKSNNYATYYADSVKDRFTISRDDSQSMLSLQMNNLKTEDTAIYYCVRGGYWSFDVWGAGTTVTVSSGGGGSGGGGSGGGGSDIVITQTTPSVPVTPGESVSISCRSSKSLLHSNGNTYLYWFLQRPGQSPQLLISRMSSLASGVPDRFSGSGSGTAFTLRISRVEAEDVGVYYCMQHLEYPYTFGGGTKLEIK

SEQ ID NO: 2 - protein, 75 aa, Artificial Sequence
  HLA-G receptor
SPTEPSSKTGNPRHLHVLIGTSVVKIPFTILLFFLLHRWCSNKKNAAVMDQEPAGNRTVNSEDSDEQDHQEVSYA

SEQ ID NO: 3 - protein, 113 aa, Artificial Sequence
  costimulatory domain
MGGLEPCSRLLLLPLLLAVSGLRPVQAQAQSDCSCSTVSPGVLAGIVMGDLVLTVLIALAVYFLGRLVPRGRGAAEAATRKQRITETESPYQELQGQRSDVYSDLNTQRPYYK

SEQ ID NO: 4 - protein, 439 aa, Artificial Sequence
  suicide protein
MGVQVETISPGDGRTFPKRGQTCVVHYTGMLEDGKKVDSSRDRNKPFKFMLGKQEVIRGWEEGVAQMSVGQRAKLTISPDYAYGATGHPGIIPPHATLVFDVELLKLESGGGSTNRQAAKLSKPTLENLTPVVLRPEIRKPEVLRPETPRPVDIGSGGFGDVGALESLRGNADLAYILSMEPCGHCLIINNVNFCRESGLRTRTGSNIDCEKLRRRFSSLHFMVEVKGDLTAKKMVLALLELAQQDHGALDCCVVVILSHGCQASHLQFPGAVYGTDGCPVSVEKIVNIFNGTSCPSLGGKPKLFFIQACGGEQKDHGFEVASTSPEDESPGSNPEPDATPFQEGLRTFDQLDAISSLPTPSDIFVSYSTFPGFVSWRDPKSGSWYVETLDDIFEQWAHSEDLQSLLLRVANAVSVKGIYKQMPGCFNFLRKKLFFKTS

SEQ ID NO: 5 - protein, 8 aa, Artificial Sequence
  CDRH1
GFTFNTYA

SEQ ID NO: 6 - protein, 10 aa, Artificial Sequence
  CDRH2
IRSKSNNYAT

SEQ ID NO: 7 - protein, 10 aa, Artificial Sequence
  CDRH3
VRGGYWSFDV

SEQ ID NO: 8 - protein, 11 aa, Artificial Sequence
  CDRL2
KSLLHSNGNTY

SEQ ID NO: 9 - protein, 9 aa, Artificial Sequence
  CDRL3
MQHLEYPYT

SEQ ID NO: 10 - protein, 22 aa, Artificial Sequence
  P2A
GSGATNFSLLKQAGDVEENPGP

SEQ ID NO: 11 - DNA, 738 bp, Artificial Sequence
  anti-HLA-G antibody coding fragment
gaggttcagctgcaagagtctggcggaggactggtgcagcctaagggaagcctgaagctgagctgtgccgccttcggcttcaccttcaacacctacgccatgcactgggtccgacaggcccctggaaaaggccttgaatgggtcgcccggatcagaagcaagagcaacaattacgccacctactacgccgacagcgtgaaggacagattcaccatcagccgggacgacagccagagcatgctgagcctgcagatgaacaacctgaaaaccgaggacaccgccatctactactgcgtcagaggcggctactggtccttcgatgtttggggagccggcaccaccgtgacagtttctagcggaggcggtggatctggcggcggaggaagtggtggcggaggttctgatatcgtgatcacccagaccacacctagcgtgccagtgacacctggcgagagcgtgtccatcagctgcagaagcagcaagagcctgctgcacagcaacggcaatacctacctgtactggttcctgcagaggcccggacagtctcctcagctgctgatctccagaatgagcagcctggctagcggcgtgcccgatagattttctggcagcggctctggcaccgccttcacactgagaatcagcagagtggaagccgaggacgtgggcgtgtactactgtatgcagcacctggaatacccctacaccttcggcggaggcaccaagctggaaatcaag

SEQ ID NO: 12 - DNA, 225 bp, Artificial Sequence
  HLA-G receptor coding fragment
tcacccactgaaccaagctccaaaaccggtaaccccagacacctgcatgttctgattgggacctcagtggtcaaaatccctttcaccatcctcctcttctttctccttcatcgctggtgctccaacaaaaaaaatgctgctgtaatggaccaagagcctgcagggaacagaacagtgaacagcgaggattctgatgaacaagaccatcaggaggtgtcatacgca

SEQ ID NO: 13 - DNA, 339 bp, Artificial Sequence
  costimulatory domain coding fragment
atggggggacttgaaccctgcagcaggctcctgctcctgcctctcctgctggctgtaagtggtctccgtcctgtccaggcccaggcccagagcgattgcagttgctctacggtgagcccgggcgtgctggcagggatcgtgatgggagacctggtgctgacagtgctcattgccctggccgtgtacttcctgggccggctggtccctcgggggcgaggggctgcggaggcagcgacccggaaacagcgtatcactgagaccgagtcgccttatcaggagctccagggtcagaggtcggatgtctacagcgacctcaacacacagaggccgtattacaaa

SEQ ID NO: 14 - DNA, 1317 bp, Artificial Sequence
  suicide gene
atgggagtgcaggtggaaaccatctccccaggagacgggcgcaccttccccaagcgcggccagacctgcgtggtgcactacaccgggatgcttgaagatggaaagaaagtggattcctcccgggacagaaacaagccctttaagtttatgctaggcaagcaggaggtgatccgaggctgggaagaaggggttgcccagatgagtgtgggtcagagagccaaactgactatatctccagattatgcctatggtgccactgggcacccaggcatcatcccaccacatgccactctcgtcttcgatgtggagcttctaaaactggaatctggaggaggttctactaacaggcaagcagcaaagttgtcgaagccaaccctagaaaaccttaccccagtggtgctcagaccagagattcgcaaaccagaggttctcagaccggaaacacccagaccagtggacattggttctggaggatttggtgatgtcggtgctcttgagagtttgaggggaaatgcagatttggcttacatcctgagcatggagccctgtggccactgcctcattatcaacaatgtgaacttctgccgtgagtccgggctccgcacccgcactggctccaacatcgactgtgagaagttgcggcgtcgcttctcctcgctgcatttcatggtggaggtgaagggcgacctgactgccaagaaaatggtgctggctttgctggagctggcgcagcaggaccacggtgctctggactgctgcgtggtggtcattctctctcacggctgtcaggccagccacctgcagttcccaggggctgtctacggcacagatggatgccctgtgtcggtcgagaagattgtgaacatcttcaatgggaccagctgccccagcctgggagggaagcccaagctctttttcatccaggcctgtggtggggagcagaaagaccatgggtttgaggtggcctccacttcccctgaagacgagtcccctggcagtaaccccgagccagatgccaccccgttccaggaaggtttgaggaccttcgaccagctggacgccatatctagtttgcccacacccagtgacatctttgtgtcctactctactttcccaggttttgtttcctggagggaccccaagagtggctcctggtacgttgagaccctggacgacatctttgagcagtgggctcactctgaagacctgcagtccctcctgcttagggtcgctaatgctgtttcggtgaaagggatttataaacagatgcctggttgctttaatttcctccggaaaaaacttttctttaaaacatca

SEQ ID NO: 15 - DNA, 66 bp, Artificial Sequence
  2A peptide coding fragment
ggatctggcgccaccaacttcagcctgctgaagcaggcaggcgacgtggaagagaaccctggccct

SEQ ID NO: 16 - DNA, 1335 bp, Artificial Sequence
  promoter
gagtaattcatacaaaaggactcgcccctgccttggggaatcccagggaccgtcgttaaactcccactaacgtagaacccagagatcgctgcgttcccgccccctcacccgcccgctctcgtcatcactgaggtggagaagagcatgcgtgaggctccggtgcccgtcagtgggcagagcgcacatcgcccacagtccccgagaagttggggggaggggtcggcaattgaaccggtgcctagagaaggtggcgcggggtaaactgggaaagtgatgtcgtgtactggctccgcctttttcccgagggtgggggagaaccgtatataagtgcagtagtcgccgtgaacgttctttttcgcaacgggtttgccgccagaacacaggtaagtgccgtgtgtggttcccgcgggcctggcctctttacgggttatggcccttgcgtgccttgaattacttccacgcccctggctgcagtacgtgattcttgatcccgagcttcgggttggaagtgggtgggagagttcgaggccttgcgcttaaggagccccttcgcctcgtgcttgagttgaggcctggcttgggcgctggggccgccgcgtgcgaatctggtggcaccttcgcgcctgtctcgctgctttcgataagtctctagccatttaaaatttttgatgacctgctgcgacgctttttttctggcaagatagtcttgtaaatgcgggccaagatctgcacactggtatttcggtttttggggccgcgggcggcgacggggcccgtgcgtcccagcgcacatgttcggcgaggcggggcctgcgagcgcggccaccgagaatcggacgggggtagtctcaagctggccggcctgctctggtgcctggcctcgcgccgccgtgtatcgccccgccctgggcggcaaggctggcccggtcggcaccagttgcgtgagcggaaagatggccgcttcccggccctgctgcagggagctcaaaatggaggacgcggcgctcgggagagcgggcgggtgagtcacccacacaaaggaaaagggcctttccgtcctcagccgtcgcttcatgtgactccacggagtaccgggcgccgtccaggcacctcgattagttctcgagcttttggagtacgtcgtctttaggttggggggaggggttttatgcgatggagtttccccacactgagtgggtggagactgaagttaggccagcttggcacttgatgtaattctccttggaatttgccctttttgagtttggatcttggttcattctcaagcctcagacagtggttcaaagtttttttcttccatttcaggtgtcgtga

SEQ ID NO: 17 - DNA, 63 bp, Artificial Sequence
  signal peptide
atggccctccctgtcaccgccctgctgcttccgctggctcttctgctccacgccgctcggccc